European Patent Application EP 4 534 681 A1, published April 9, 2025. Title: ウイルスベクター及びそれを含むがん細胞増殖抑制剤. Applicant: HIKARI BIO Inc. Application JP 2022-88235, filed May 31, 2022. The sequence listing filed with the application follows.

SEQUENCE LISTING (40 sequences)

SEQ ID NO: 1 - DNA, 25 bp, Homo sapiens
  source 1..25: mol_type = genomic DNA
ccagtactcccggcccccgccattt

SEQ ID NO: 2 - DNA, 26 bp, Homo sapiens
  source 1..26: mol_type = genomic DNA
cggactgggagcgagcgcggcgcagg

SEQ ID NO: 3 - DNA, 17 bp, Homo sapiens
  source 1..17: mol_type = genomic DNA
ggacactttgcgttcgg

SEQ ID NO: 4 - DNA, 20 bp, Homo sapiens
  source 1..20: mol_type = genomic DNA
gctgggagcgtgctttccac

SEQ ID NO: 5 - DNA, 17 bp, Homo sapiens
  source 1..17: mol_type = genomic DNA
aatgactgaatataaac

SEQ ID NO: 6 - DNA, 21 bp, Homo sapiens
  source 1..21: mol_type = genomic DNA
ttgtggtagttggagctggtg

SEQ ID NO: 7 - DNA, 17 bp, Homo sapiens
  source 1..17: mol_type = genomic DNA
cacttttcgacatagtg

SEQ ID NO: 8 - DNA, 24 bp, Homo sapiens
  source 1..24: mol_type = genomic DNA
tggtggtgccctatgagccgcctg

SEQ ID NO: 9 - DNA, 17 bp, Homo sapiens
  source 1..17: mol_type = genomic DNA
ccacgggtgtattgtgt

SEQ ID NO: 10 - DNA, 20 bp, Homo sapiens
  source 1..20: mol_type = genomic DNA
gacacctataaacttttcca

SEQ ID NO: 11 - DNA, 35 bp, synthetic construct
  source 1..35: mol_type = other DNA
ggcggctcggccagtactcccggcccccgccattt

SEQ ID NO: 12 - DNA, 30 bp, synthetic construct
  source 1..30: mol_type = other DNA
ccgactgggagcgagcgcggcgcaggcact

SEQ ID NO: 13 - DNA, 30 bp, synthetic construct
  source 1..30: mol_type = other DNA
tgctgggctccggggacactttgcgttccg

SEQ ID NO: 14 - DNA, 30 bp, synthetic construct
  source 1..30: mol_type = other DNA
gctgggagcgtgctttccacgacggtgaca

SEQ ID NO: 15 - DNA, 27 bp, synthetic construct
  source 1..27: mol_type = other DNA
gcctgctgaaaatgactgaatatatac

SEQ ID NO: 16 - DNA, 30 bp, synthetic construct
  source 1..30: mol_type = other DNA
ttgtggtagttggagctggtggcgtaggca

SEQ ID NO: 17 - DNA, 30 bp, synthetic construct
  source 1..30: mol_type = other DNA
tggatgacagaaacacttttcgacatagtg

SEQ ID NO: 18 - DNA, 26 bp, synthetic construct
  source 1..26: mol_type = other DNA
tcgtggtgccctatgagccgcctgag

SEQ ID NO: 19 - DNA, 30 bp, synthetic construct
  source 1..30: mol_type = other DNA
tttgacaatatagacaatttaagtcccacg

SEQ ID NO: 20 - DNA, 30 bp, synthetic construct
  source 1..30: mol_type = other DNA
gcatctcatcgtagtaagcagagacacaag

SEQ ID NO: 21 - DNA, 17 bp, Homo sapiens
  source 1..17: mol_type = genomic DNA
aatgactgaatataaac

SEQ ID NO: 22 - DNA, 21 bp, Homo sapiens
  source 1..21: mol_type = genomic DNA
ttgtggtagttggagctggtg

SEQ ID NO: 23 - DNA, 16 bp, Homo sapiens
  source 1..16: mol_type = genomic DNA
gacactttgcgttcgg

SEQ ID NO: 24 - DNA, 20 bp, Homo sapiens
  source 1..20: mol_type = genomic DNA
gctgggagcgtgctttccac

SEQ ID NO: 25 - DNA, 17 bp, Homo sapiens
  source 1..17: mol_type = genomic DNA
aatgactgaatataaac

SEQ ID NO: 26 - DNA, 21 bp, Homo sapiens
  source 1..21: mol_type = genomic DNA
ttgtggtagttggagctggtg

SEQ ID NO: 27 - DNA, 17 bp, Homo sapiens
  source 1..17: mol_type = genomic DNA
cacttttcgacatagtg

SEQ ID NO: 28 - DNA, 24 bp, Homo sapiens
  source 1..24: mol_type = genomic DNA
tggtggtgccctatgagccgcctg

SEQ ID NO: 29 - DNA, 17 bp, Homo sapiens
  source 1..17: mol_type = genomic DNA
ccacgggtgtattgtgt

SEQ ID NO: 30 - DNA, 20 bp, Homo sapiens
  source 1..20: mol_type = genomic DNA
gacacctataaacttttcca

SEQ ID NO: 31 - DNA, 648 bp, synthetic construct
  source 1..648: mol_type = other DNA
gagtcgacggcggctcggccagtactcccggcccccgccatttatgactgaatataaacttgtggtagttggagctggtggcgtaggcaagagtgccttgacgatacagctaattcagaatcattttgtggacgaatatgatccaacaatagaggattcctacaggaagcaagtagtaattgatggagaaacctgtctcttggatattctcgacacagcaggtcatgaggagtacagtgcaatgagggaccagtacatgaggactggggagggctttctttgtgtatttgccataaataatactaaatcatttgaagatattcaccattatagagaacaaattaaaagagttaaggactctgaagatgtacctatggtcctagtaggaaataaatgtgatttgccttctagaacagtagacacaaaacaggctcaggacttagcaagaagttatggaattccttttattgaaacatcagcaaagacaagacagggtgttgatgatgccttctatacattagttcgagaaattcgaaaacataaagaaaagatgagcaaagatggtaaaaagaagaaaaagaagtcaaagacaaagtgtgtaattatgtagcggactgggagcgagcgcggcgcaggcactggatccaa

SEQ ID NO: 32 - DNA, 605 bp, synthetic construct
  source 1..605: mol_type = other DNA
gagtcgacaatgactgaatataaacttgtggtagttggagctggtggcgtaggcaagagtgccttgacgatacagctaattcagaatcattttgtggacgaatatgatccaacaatagaggattcctacaggaagcaagtagtaattgatggagaaacctgtctcttggatattctcgacacagcaggtcatgaggagtacagtgcaatgagggaccagtacatgaggactggggagggctttctttgtgtatttgccataaataatactaaatcatttgaagatattcaccattatagagaacaaattaaaagagttaaggactctgaagatgtacctatggtcctagtaggaaataaatgtgatttgccttctagaacagtagacacaaaacaggctcaggacttagcaagaagttatggaattccttttattgaaacatcagcaaagacaagacagggtgttgatgatgccttctatacattagttcgagaaattcgaaaacataaagaaaagatgagcaaagatggtaaaaagaagaaaaagaagtcaaagacaaagtgtgtaattatgtagttgtggtagttggagctggtgggatccaa

SEQ ID NO: 33 - DNA, 1257 bp, synthetic construct
  source 1..1257: mol_type = other DNA
agaattctgctgggctccggggacactttgcgttcggatggaggagccgcagtcagatcctagcgtcgagccccctctgagtcaggaaacattttcagacctatggaaactacttcctgaaaacaacgttctgtcccccttgccgtcccaagcaatggatgatttgatgctgtccccggacgatattgaacaatggttcactgaagacccaggtccagatgaagctcccagaatgccagaggctgctccccccgtggcccctgcaccagcagctcctacaccggcggcccctgcaccagccccctcctggcccctgtcatcttctgtcccttcccagaaaacctaccagggcagctacggtttccgtctgggcttcttgcattctgggacagccaagtctgtgacttgcacgtactcccctgccctcaacaagatgttttgccaactggccaagacctgccctgtgcagctgtgggttgattccacacccccgcccggcacccgcgtccgcgccatggccatctacaagcagtcacagcacatgacggaggttgtgaggcgctgcccccaccatgagcgctgctcagatagcgatggtctggcccctcctcagcatcttatccgagtggaaggaaatttgcgtgtggagtatttggatgacagaaacacttttcgacatagtgtggtggtgccctatgagccgcctgaggttggctctgactgtaccaccatccactacaactacatgtgtaacagttcctgcatgggcggcatgaaccggaggcccatcctcaccatcatcacactggaagactccagtggtaatctactgggacggaacagctttgaggtgcgtgtttgtgcctgtcctgggagagaccggcgcacagaggaagagaatctccgcaagaaaggggagcctcaccacgagctgcccccagggagcactaagcgagcactgcccaacaacaccagctcctctccccagccaaagaagaaaccactggatggagaatatttcacccttcagatccgtgggcgtgagcgcttcgagatgttccgagagctgaatgaggccttggaactcaaggatgcccaggctgggaaggagccaggggggagcagggctcactccagccacctgaagtccaaaaagggtcagtctacctcccgccataaaaaactcatgttcaagacagaagggcctgactcagactgagctgggagcgtgctttccacgacggtgacaggatccaa

SEQ ID NO: 34 - DNA, 609 bp, synthetic construct
  source 1..609: mol_type = other DNA
agaattccacttttcgacatagtgcacttttcgacatagtgtggtggtgccctatgagccgcctgaggttggctctgactgtaccaccatccactacaactacatgtgtaacagttcctgcatgggcggcatgaaccggaggcccatcctcaccatcatcacactggaagactccagtggtaatctactgggacggaacagctttgaggtgcgtgtttgtgcctgtcctgggagagaccggcgcacagaggaagagaatctccgcaagaaaggggagcctcaccacgagctgcccccagggagcactaagcgagcactgcccaacaacaccagctcctctccccagccaaagaagaaaccactggatggagaatatttcacccttcagatccgtgggcgtgagcgcttcgagatgttccgagagctgaatgaggccttggaactcaaggatgcccaggctgggaaggagccaggggggagcagggctcactccagccacctgaagtccaaaaagggtcagtctacctcccgccataaaaaactcatgttcaagacagaagggcctgactcagactgatggtggtgccctatgagccgcctgggatccaa

SEQ ID NO: 35 - DNA, 3653 bp, synthetic construct
  source 1..3653: mol_type = other DNA
agaattcccacgggtgtattgtgttgaagggacacctataaacttttccacagctacatctctaagtgatctaacaatcgaatcccctccaaatgagttagctgctggagaaggagttagaggaggggcacagtcaggtgaatttgaaaaacgagataccattcctacagaaggcagaagtacagatgaggctcaaggaggaaaaacctcatctgtaaccatacctgaattggatgacaataaagcagaggaaggtgatattcttgcagaatgcattaattctgctatgcccaaagggaaaagtcacaagcctttccgtgtgaaaaagataatggaccaggtccagcaagcatctgcgtcttcttctgcacccaacaaaaatcagttagatggtaagaaaaagaaaccaacttcaccagtaaaacctataccacaaaatactgaatataggacacgtgtaagaaaaaatgcagactcaaaaaataatttaaatgctgagagagttttctcagacaacaaagattcaaagaaacagaatttgaaaaataattccaaggtcttcaatgataagctcccaaataatgaagatagagtcagaggaagttttgcttttgattcacctcatcattacacgcctattgaaggaactccttactgtttttcacgaaatgattctttgagttctctagattttgatgatgatgatgttgacctttccagggaaaaggctgaattaagaaaggcaaaagaaaataaggaatcagaggctaaagttaccagccacacagaactaacctccaaccaacaatcagctaataagacacaagctattgcaaagcagccaataaatcgaggtcagcctaaacccatacttcagaaacaatccacttttccccagtcatccaaagacataccagacagaggggcagcaactgatgaaaagttacagaattttgctattgaaaatactccggtttgcttttctcataattcctctctgagttctctcagtgacattgaccaagaaaacaacaataaagaaaatgaacctatcaaagagactgagccccctgactcacagggagaaccaagtaaacctcaagcatcaggctatgctcctaaatcatttcatgttgaagataccccagtttgtttctcaagaaacagttctctcagttctcttagtattgactctgaagatgacctgttgcaggaatgtataagctccgcaatgccaaaaaagaaaaagccttcaagactcaagggtgataatgaaaaacatagtcccagaaatatgggtggcatattaggtgaagatctgacacttgatttgaaagatatacagagaccagattcagaacatggtctatcccctgattcagaaaattttgattggaaagctattcaggaaggtgcaaattccatagtaagtagtttacatcaagctgctgctgctgcatgtttatctagacaagcttcgtctgattcagattccatcctttccctgaaatcaggaatctctctgggatcaccatttcatcttacacctgatcaagaagaaaaaccctttacaagtaataaaggcccacgaattctaaaaccaggggagaaaagtacattggaaactaaaaagatagaatctgaaagtaaaggaatcaaaggaggaaaaaaagtttataaaagtttgattactggaaaagttcgatctaattcagaaatttcaggccaaatgaaacagccccttcaagcaaacatgccttcaatctctcgaggcaggacaatgattcatattccaggagttcgaaatagctcctcaagtacaagtcctgtttctaaaaaaggcccaccccttaagactccagcctccaaaagccctagtgaaggtcaaacagccaccacttctcctagaggagccaagccatctgtgaaatcagaattaagccctgttgccaggcagacatcccaaataggtgggtcaagtaaagcaccttctagatcaggatctagagattcgaccccttcaagacctgcccagcaaccattaagtagacctatacagtctcctggccgaaactcaatttcccctggtagaaatggaataagtcctcctaacaaattatctcaacttccaaggacatcatcccctagtactgcttcaactaagtcctcaggttctggaaaaatgtcatatacatctccaggtagacagatgagccaacagaaccttaccaaacaaacaggtttatccaagaatgccagtagtattccaagaagtgagtctgcctccaaaggactaaatcagatgaataatggtaatggagccaataaaaaggtagaactttctagaatgtcttcaactaaatcaagtggaagtgaatctgatagatcagaaagacctgtattagtacgccagtcaactttcatcaaagaagctccaagcccaaccttaagaagaaaattggaggaatctgcttcatttgaatctctttctccatcatctagaccagcttctcccactaggtcccaggcacaaactccagttttaagtccttcccttcctgatatgtctctatccacacattcgtctgttcaggctggtggatggcgaaaactcccacctaatctcagtcccactatagagtataatgatggaagaccagcaaagcgccatgatattgcacggtctcattctgaaagtccttctagacttccaatcaataggtcaggaacctggaaacgtgagcacagcaaacattcatcatcccttcctcgagtaagcacttggagaagaactggaagttcatcttcaattctttctgcttcatcagaatccagtgaaaaagcaaaaagtgaggatgaaaaacatgtgaactctatttcaggaaccaaacaaagtaaagaaaaccaagtatccgcaaaaggaacatggagaaaaataaaagaaaatgaattttctcccacaaatagtacttctcagaccgtttcctcaggtgctacaaatggtgctgaatcaaagactctaatttatcaaatggcacctgctgtttctaaaacagaggatgtttgggtgagaattgaggactgtcccattaacaatcctagatctggaagatctcccacaggtaatactcccccggtgattgacagtgtttcagaaaaggcaaatccaaacattaaagattcaaaagataatcaggcaaaacaaaatgtgggtaatggcagtgttcccatgcgtaccgtgggtttggaaaatcgcctgaactcctttattcaggtggatgcccctgaccaaaaaggaactgagataaaaccaggacaaaataatcctgtccctgtatcagagactaatgaaagttctatagtggaacgtaccccattcagttctagcagctcaagcaaacacagttcacctagtgggactgttgctgccagagtgactccttttaattacaacccaagccctaggaaaagcagcgcagatagcacttcagctcggccatctcagatcccaactccagtgaataacaacacaaagaagcgagattccaaaactgacagcacagaatccagtggaacccaaagtcctaagcgccattctgggtcttaccttgtgacatctgtttaagacacctataaacttttccaggatccaa

SEQ ID NO: 36 - DNA, 122 bp, Homo sapiens
  source 1..122: mol_type = genomic DNA
gcctgctgaaaatgactgaatataaacttgtggtagttggagctggtggcgtaggcaagagtgccttgacgatacagctaattcagaatcattttgtggacgaatatgatccaacaatagag

SEQ ID NO: 37 - DNA, 174 bp, Homo sapiens
  source 1..174: mol_type = genomic DNA
gatgggattggggttttcccctcccatgtgctcaagactggcgctaaaagttttgagcttctcaaaagtctagagccaccgtccagggagcaggtagctgctgggctccggggacactttgcgttcgggctgggagcgtgctttccacgacggtgacacgcttccctggattgg

SEQ ID NO: 38 - DNA, 106 bp, Homo sapiens
  source 1..106: mol_type = genomic DNA
ccagtactcccggcccccgccatttcggactgggagcgagcgcggcgcaggcactgaaggcggcggcggggccagaggctcagcggctcccaggtgcgggagagag

SEQ ID NO: 39 - DNA, 112 bp, Homo sapiens
  source 1..112: mol_type = genomic DNA
cacttttcgacatagtgtggtggtgccctatgagccgcctgaggttggctctgactgtaccaccatccactacaactacatgtgtaacagttcctgcatgggcggcatgaac

SEQ ID NO: 40 - DNA, 121 bp, Homo sapiens
  source 1..121: mol_type = genomic DNA
ccacgggtgtattgtgtgacacctataaacttttccacagctacatctctaagtgatctaacaatcgaatcccctccaaatgagttagctgctggagaaggagttagaggaggggcacagt